European Patent Application EP 4 591 702 A2, published July 30, 2025. Title: METHODS AND COMPOSITIONS FOR PRODUCING CAPSICUM PLANTS WITH POWDERY MILDEW RESISTANCE. Applicant: SEMINIS VEGETABLE SEEDS, INC. Application EP EP 12827559.1, filed August 29, 2012. The sequence listing filed with the application follows.

SEQUENCE LISTING (44 sequences)

SEQ ID NO: 1 - DNA, 121 bp, synthetic construct
  misc_feature 1..121: note = Synthetic primer
  source 1..121: mol_type = other DNA
atactaaatccaatagtgctcttccgctgaaagttcataatagcctgtagatttgaaagargcaagaggttaatccaaatgaattcgcgatgaaaagcagaataaacgaaacccgggactt

SEQ ID NO: 2 - DNA, 121 bp, synthetic construct
  misc_feature 1..121: note = Synthetic primer
  source 1..121: mol_type = other DNA
aataatttatagctccacaaatagtcgataagtggtttagatcaaaaagttgaaaagtctytcttacactttgtgccaagtcaaaggcagtggcggatctacatacaattcaaggggttca

SEQ ID NO: 3 - DNA, 121 bp, synthetic construct
  misc_feature 1..121: note = Synthetic primer
  source 1..121: mol_type = other DNA
aattccattagaacaggttccatcagagcagcaaaagattgttcaactatgcaggcagctraataggcctgttatagttgcttcccagttgctggaatctatgattgaataccctattccc

SEQ ID NO: 4 - DNA, 107 bp, synthetic construct
  misc_feature 1..107: note = Synthetic primer
  misc_feature 92..93: note = n is a, c, g, or t
  source 1..107: mol_type = other DNA
caatttgcaagggaaaatccagcctccatgatgacttatcacaggtcgtaaacactgtgtrgtcaatgtagaaactgtaaaaaaaaaaaaanncattaactagacaa

SEQ ID NO: 5 - DNA, 120 bp, synthetic construct
  misc_feature 1..120: note = Synthetic primer
  source 1..120: mol_type = other DNA
gagatcaaatgattcagacaaataaagaatactaaaagaaagtaacatacagtaagagamacatgtgaaacaatgtaagacaattaagagaagggtgagaaagcccacccctccacgtgc

SEQ ID NO: 6 - DNA, 121 bp, synthetic construct
  misc_feature 1..121: note = Synthetic primer
  misc_feature 4: note = n is a, c, g, or t
  source 1..121: mol_type = other DNA
tgangtctttgggtaggaatcctaaatagaaatttgtgcagtggagaagtacgtcctgtcraaggaattgggaagtcactgagtgtcggacaagttgtatgggctccatctggtgaaggct

SEQ ID NO: 7 - DNA, 121 bp, synthetic construct
  misc_feature 1..121: note = Synthetic primer
  source 1..121: mol_type = other DNA
gtaactgacgtaagggtagatccaagatttgaacattatgtattcgagttagactttctaktgtagtccatttggtttatttatgactcgaaacctattatttgcactcgtttagtaaaca

SEQ ID NO: 8 - DNA, 121 bp, synthetic construct
  misc_feature 1..121: note = Synthetic primer
  source 1..121: mol_type = other DNA
cgttccaagtaccaactcatccacacagtacgtacacacaagggcgtggatgaaaggagcwatggctgtgtgttccgggaggaggaagagaaggaggaggtaggcgttgccctgtcgaagg

SEQ ID NO: 9 - DNA, 120 bp, synthetic construct
  misc_feature 1..120: note = Synthetic primer
  source 1..120: mol_type = other DNA
gccttcggaaatccaaatgtgcctggtgctggttatggtagcggtcaagctggtggatcragaagctcgtggggttctcagggtccttctggatatgggaacatgggctatggtaatgca

SEQ ID NO: 10 - DNA, 121 bp, synthetic construct
  misc_feature 1..121: note = Synthetic primer
  source 1..121: mol_type = other DNA
gtggtatgggtggtggaagttaccaggggtatggtgcatctggtgacaatcccagttcttrtgacagaatggataccaacagatacatgcagtcacaaaacactgtaggtggctatccacc

SEQ ID NO: 11 - DNA, 117 bp, synthetic construct
  misc_feature 1..117: note = Synthetic primer
  source 1..117: mol_type = other DNA
gccatagttaaataggttctccttctgctaatgtacatcatctatgaaatttaacatctgyataatgcaggtgcctcctactttgagatttgtgatggatggtgaaatgcccgatta

SEQ ID NO: 12 - DNA, 121 bp, synthetic construct
  misc_feature 1..121: note = Synthetic primer
  misc_feature 23: note = n is a, c, g, or t
  misc_feature 37: note = n is a, c, g, or t
  misc_feature 41: note = n is a, c, g, or t
  source 1..121: mol_type = other DNA
cacacaaccgatacttactattncagaaagtcacttncttngcaaccctccggggaagttrgtcactttgtcaatcagaaatgcagaatttaaccaagaataccaagcggccgtttcctca

SEQ ID NO: 13 - DNA, 121 bp, synthetic construct
  misc_feature 1..121: note = Synthetic primer
  source 1..121: mol_type = other DNA
gatataggagtatcatggaagttgtgccctttgatatggtatgcgtggaaccatttgatcyacatttgtccagtttatgctctaagtcccagcatatcttagcaatagcagccctgttaca

SEQ ID NO: 14 - DNA, 102 bp, synthetic construct
  misc_feature 1..102: note = Synthetic primer
  source 1..102: mol_type = other DNA
ctattgggaagcctcccaccaaacatatgttctatcttacccaacgttgaaagcgtttatytggcctataccaattttgctgggactattcctcattccatc

SEQ ID NO: 15 - DNA, 121 bp, synthetic construct
  misc_feature 1..121: note = Synthetic primer
  misc_feature 26: note = n is a, c, g, or t
  source 1..121: mol_type = other DNA
acagaattggtagccttgatcacccngcttcgggtcctggtgacatggtggaacatttgcrgccagaaactgagtcatttactgaggttttacttgcaaagtttgtccgaatgctccagaa

SEQ ID NO: 16 - DNA, 121 bp, synthetic construct
  misc_feature 1..121: note = Synthetic primer
  misc_feature 14..15: note = n is a, c, g, or t
  misc_feature 23: note = n is a, c, g, or t
  misc_feature 30: note = n is a, c, g, or t
  source 1..121: mol_type = other DNA
tgacctttatagtnnaaaaaaanttaaaanggacaagaaatggaaagggaacaaagaagartatcagcagcttatctatgtttaacaaattatgacctccattagcttttatattaataaa

SEQ ID NO: 17 - DNA, 121 bp, synthetic construct
  misc_feature 1..121: note = Synthetic primer
  misc_feature 90: note = n is a, c, g, or t
  misc_feature 107: note = n is a, c, g, or t
  source 1..121: mol_type = other DNA
cgatacatgcgcaccactcgacatcttttgtggttctcaagataacaatcgcaggtaacakcatctgtaaatccaatagaacaacttggnggtaataatattccctnagaacacccaagca

SEQ ID NO: 18 - DNA, 121 bp, synthetic construct
  misc_feature 1..121: note = Synthetic primer
  source 1..121: mol_type = other DNA
tggaatcaagggtcaggaagactgaaatgttgtatgccgaaggtcgtcagctgaaagtgartctaagtcttttaatacttagaaaaattttcatacttttcaagactaagtgcactctact

SEQ ID NO: 19 - DNA, 121 bp, synthetic construct
  misc_feature 1..121: note = Synthetic primer
  misc_feature 2: note = n is a, c, g, or t
  misc_feature 12: note = n is a, c, g, or t
  misc_feature 113: note = n is a, c, g, or t
  source 1..121: mol_type = other DNA
cngggttggggnaagggctgaatcttatagttctttctgtgtgtcaagttaacgcctcgtrgagtcacttacgatctcttcgtttccatttttcttcttgttaaagaatgaanttgggtct

SEQ ID NO: 20 - DNA, 121 bp, synthetic construct
  misc_feature 1..121: note = Synthetic primer
  source 1..121: mol_type = other DNA
aaaattgccttagtacgaattaatactcttatatattctcaaaagacatatacccagaccrtacttgtgggattacaccggctatgttgtggttgttttgtgaagacatatttaagtactc

SEQ ID NO: 21 - DNA, 121 bp, synthetic construct
  misc_feature 1..121: note = Synthetic primer
  misc_feature 26: note = n is a, c, g, or t
  misc_feature 34..35: note = n is a, c, g, or t
  source 1..121: mol_type = other DNA
gttaagcttctgtgaagccaaaagtntttttttnncgaagtgtttagttaaaaaagttgcrttgtttggccaagcttttaggaaaaagataagtatttcgagtcgttgtagaaactgcact

SEQ ID NO: 22 - DNA, 121 bp, synthetic construct
  misc_feature 1..121: note = Synthetic primer
  source 1..121: mol_type = other DNA
ctgttcaagagcaattcagtcatttgttcttcaggtaatcttgtttattcccaaattgtgscaatcaatttggttctcatcattggtatcagagacctaatcatctgacctgtgcgatggg

SEQ ID NO: 23 - DNA, 121 bp, synthetic construct
  misc_feature 1..121: note = Synthetic primer
  misc_feature 6: note = n is a, c, g, or t
  misc_feature 108: note = n is a, c, g, or t
  source 1..121: mol_type = other DNA
tacacnggtaaaactgacaaggcatcagcgttagccaataatgaacttttagcgcggaacytcaagtgaccaagtgcatgaaaccaaatcaagaaggtaaagatatgntgatcacctgaat

SEQ ID NO: 24 - DNA, 121 bp, synthetic construct
  misc_feature 1..121: note = Synthetic primer
  source 1..121: mol_type = other DNA
tggatataggaaagatcacttagaaattcaacaatctttttcgtctttaagagcctgtagrcttctttagcatctacacatcaaaattctccagacatttcaaattatatacagtccacga

SEQ ID NO: 25 - DNA, 121 bp, synthetic construct
  misc_feature 1..121: note = Synthetic primer
  source 1..121: mol_type = other DNA
actcttttattcgtaatgttcatagacgaaagagacgatccttcgctcctgtgagcaggayggtgttccaatgtgcaaggccctttcctgaagaggtcgaaaattcacgacccattcatag

SEQ ID NO: 26 - DNA, 113 bp, synthetic construct
  misc_feature 1..113: note = Synthetic primer
  misc_feature 93: note = n is a, c, g, or t
  source 1..113: mol_type = other DNA
taagtacaagtttaaggattcaagttatctcttaaattagctttcagaacatgatgacatkctttctgctttgcgatgggacagatggaatantcaagtcatgttgacttgat

SEQ ID NO: 27 - DNA, 121 bp, synthetic construct
  misc_feature 1..121: note = Synthetic primer
  source 1..121: mol_type = other DNA
aataatgacattcgatttgtcagcaactaaatcaaagcactccatcaagcaacaataagakatccggactttcatccgcatgcaccctcacagcaagaaagttccccatactacttacact

SEQ ID NO: 28 - DNA, 119 bp, synthetic construct
  misc_feature 1..119: note = Synthetic primer
  source 1..119: mol_type = other DNA
gtttttccaatgtatccaccaaatacagtcatgccttttgtatattgggatcaacctartgtgttcgcgccagttcattatcgctcttcttatagatgtatcgcacctggaagttgcat

SEQ ID NO: 29 - DNA, 121 bp, synthetic construct
  misc_feature 1..121: note = Synthetic primer
  misc_feature 15: note = n is a, c, g, or t
  misc_feature 22: note = n is a, c, g, or t
  source 1..121: mol_type = other DNA
ctttttctcttattnccttttnattttcttgttttgctactaaaagcttgaagttctattktgcaatgtgcatacttgcttgaagtctcgtattcacatgttaagaccttctctttagaaa

SEQ ID NO: 30 - DNA, 121 bp, synthetic construct
  misc_feature 1..121: note = Synthetic primer
  misc_feature 28: note = n is a, c, g, or t
  source 1..121: mol_type = other DNA
cttagatcaaaagtgaatacaacaaaangttaccggatgattccatttctaagccgaccayatccacagtaaacccatatgtagcaagatagaaattgaaaacaattatcaccgtacacat

SEQ ID NO: 31 - DNA, 121 bp, synthetic construct
  misc_feature 1..121: note = Synthetic primer
  source 1..121: mol_type = other DNA
gcgcccacgaacattgccgtgttgggagttaccaagaggctgatgcagaatgtacaaagtygtctgcaatacgacacgtatggttttggagacattgtcttatttggtaacggggagagaa

SEQ ID NO: 32 - DNA, 121 bp, synthetic construct
  misc_feature 1..121: note = Synthetic primer
  source 1..121: mol_type = other DNA
ctcgtcttctttcttgatcttttaagcaccgcgttgatgaaatttttcgtgttttgcttayacgagttgcatttttgaaataatgttagtacgttttcagattatgatcatagacttcaaa

SEQ ID NO: 33 - DNA, 121 bp, synthetic construct
  misc_feature 1..121: note = Synthetic primer
  misc_feature 85: note = n is a, c, g, or t
  misc_feature 94: note = n is a, c, g, or t
  misc_feature 108: note = n is a, c, g, or t
  source 1..121: mol_type = other DNA
aatagatcaaatcaacaatggagtttaattgagaaaaagaagaagccaataacagatatcrcacaaatttggattagaatcgagnagaatgagnacatagatcacacnaattcctcagaat

SEQ ID NO: 34 - DNA, 121 bp, synthetic construct
  misc_feature 1..121: note = Synthetic primer
  source 1..121: mol_type = other DNA
ggggcggagctagagttgtagttacggatttagcagaacgaatgacacttctatagggctyaagtagttggaatgaatcagttactactgatcaaagttatcaaaagttttcgtattgtct

SEQ ID NO: 35 - DNA, 121 bp, synthetic construct
  misc_feature 1..121: note = Synthetic primer
  source 1..121: mol_type = other DNA
cttaagaacactcccacttcggcttaagcaccatcgaaaagacaaactagaaccagctcaygcatacaataaaaagcatacacaaaagttacgaaccataattggtcgtaaaatggagcag

SEQ ID NO: 36 - DNA, 121 bp, synthetic construct
  misc_feature 1..121: note = Synthetic primer
  misc_feature 83: note = n is a, c, g, or t
  source 1..121: mol_type = other DNA
tcttggaaaatcgatatcagaaatggaaatcccatcgggctgtcaggagttgactcttagytatctttgtgaaagttccaaantggggtttggagagagagatgttttcgtggataaaggt

SEQ ID NO: 37 - DNA, 121 bp, synthetic construct
  misc_feature 1..121: note = Synthetic primer
  misc_feature 75: note = n is a, c, g, or t
  source 1..121: mol_type = other DNA
cttaagaacactcccacttcggcttaagcaccatcgaaaagacaaactagaaccagctcaygcatacaataaaangcatacacaaaagttacgaaccataattggtcgtaaaatggagcag

SEQ ID NO: 38 - DNA, 121 bp, synthetic construct
  misc_feature 1..121: note = Synthetic primer
  source 1..121: mol_type = other DNA
ctttatcgatgattatctgctctggaggtgtacgtttctcaacagtttctatacttgcaayagttaggcttgatgttgttaaagcctaactactcgcaaacacactcagaaccaaatgcaa

SEQ ID NO: 39 - DNA, 121 bp, synthetic construct
  misc_feature 1..121: note = Synthetic primer
  misc_feature 88: note = n is a, c, g, or t
  misc_feature 110: note = n is a, c, g, or t
  misc_feature 117: note = n is a, c, g, or t
  source 1..121: mol_type = other DNA
atcggcatcctcaagactatccattgttataaaagcaaaaccacgagagatacgagaacgyggctccacaaccaagaaagctgatttnacctggtcgacagaaagtaaangaaaaanctca

SEQ ID NO: 40 - DNA, 121 bp, synthetic construct
  misc_feature 1..121: note = Synthetic primer
  source 1..121: mol_type = other DNA
cagatattttcagtaaaatcgtaattagatccttgagatctaactgcactctaatgtcacytcaggaggcaaaaccaaagaagattttttcttccagctccattaactaaaccgcatactc

SEQ ID NO: 41 - DNA, 292 bp, synthetic construct
  misc_feature 1..292: note = Synthetic primer
  misc_feature 105: note = n is a, c, g, or t
  misc_feature 138..139: note = n is a, c, g, or t
  misc_feature 143: note = n is a, c, g, or t
  misc_feature 184: note = n is a, c, g, or t
  misc_feature 259: note = n is a, c, g, or t
  source 1..292: mol_type = other DNA
caaccatccctcaactaacgtgggacacttaacaatctaccgcacacccaggcccgcctactagagcgtggacgaaataatgagggccctacatggagacgcacngtaagagggatgagtctggctctgaccatgtgnntaantcaatcctaaaagctatctcatgaagtgaggattgaccacnaccatacaacragctacaaacaagccatccctcaaccaatatgggacattaaacacttcttaagttccaacttanaagtgttgtcttgaaggattgagcaagtgtcaa

SEQ ID NO: 42 - DNA, 218 bp, synthetic construct
  misc_feature 1..218: note = Synthetic primer
  misc_feature 22: note = n is a, c, g, or t
  misc_feature 107: note = n is a, c, g, or t
  source 1..218: mol_type = other DNA
atgcatgagggcaatacaagcnttgaatcgaaatgactgtttaatctcgtggactgtatataatttgaaatgtctggagaattttgatgtgtagatgctaaagaagnctacaggctcytaaagacgaaaaagattgttgaatttctaagtgatctttcctatatccacccctaagctgccagcgctgggggttcctttctcttggttggccttcctag

SEQ ID NO: 43 - DNA, 252 bp, synthetic construct
  misc_feature 1..252: note = Synthetic primer
  misc_feature 157: note = n is a, c, g, or t
  misc_feature 172: note = n is a, c, g, or t
  source 1..252: mol_type = other DNA
ccgttttaacatatgtacatggcttgtcttagttactaatatcatctgataccatgtgcaaacatgacttgggaatgtgggacttaatatacttgtaaccmtgtgttttgttattgaaattaaagttcagtgttatgtttgtttaaaacggccactnggtacatgttatacngctcttggtctaagctcttatctacatactataaataactttttttgttcttggtttctatcaccaattattattttatc

SEQ ID NO: 44 - DNA, 184 bp, synthetic construct
  misc_feature 1..184: note = Synthetic primer
  misc_feature 109: note = n is a, c, g, or t
  misc_feature 121: note = n is a, c, g, or t
  source 1..184: mol_type = other DNA
atttctggatttctacttgtaaaagggaagcccggtgcactaaagcgcccgttatgcaagggggccggggaaggttcagcctgcaacggtccattgtacgyagccttancctgcatttctncaagaggctgtttccacagcttgaatccgtgacctcctggtcacatggcaacaactttaccca